European Patent Specification EP 4 005 585 B1, published March 27, 2024. Title: COMPOSITIONS AND METHODS FOR TREATING PULMONARY HYPERTENSION. Applicant: THE BRIGHAM AND WOMEN'S HOSPITAL, INC. ACCELERON PHARMA INC. Application PCT/US14/667766. The sequence listing filed with the application follows.

SEQUENCE LISTING (79 sequences)

SEQ ID NO: 1 - protein, 364 aa, Artificial Sequence
  Description of Artificial Sequence: Synthetic polypeptide
TIPPHVQKSVNNDMIVTDNNGAVKFPQLCKFCDVRFSTCDNQKSCMSNCSITSICEKPQEVCVAVWRKNDENITLETVCHDPKLPYHDFILEDAASPKCIMKEKKKPGETFFMCSCSSDECNDNIIFSEEYNTSNPDTGGGVECPPCPAPPVAGPSVFLFPPKPKDTLMISRTPEVTCVVVDVSHEDPEVQFNWYVDGVEVHNAKTKPREEQFNSTFRVVSVLTVVHQDWLNGKEYKCKVSNKGLPAPIEKTISKTKGQPREPQVYTLPPSREEMTKNQVSLTCLVKGFYPSDIAVEWESNGQPENNYKTTPPMLDSDGSFFLYSKLTVDKSRWQQGNVFSCSVMHEALHNHYTQKSLSLSPGK

SEQ ID NO: 2 - DNA, 1164 bp, Artificial Sequence
  Description of Artificial Sequence: Synthetic polynucleotide
atggatgcaatgaagagagggctctgctgtgtgctgctgctgtgtggagcagtcttcgtttcgcccggcgccacgatcccaccgcacgttcagaagtcggttaataacgacatgatagtcactgacaacaacggtgcagtcaagtttccacaactgtgtaaattttgtgatgtgagattttccacctgtgacaaccagaaatcctgcatgagcaactgcagcatcacctccatctgtgagaagccacaggaagtctgtgtggctgtatggagaaagaatgacgagaacataacactagagacagtttgccatgaccccaagctcccctaccatgactttattctggaagatgctgcttctccaaagtgcattatgaaggaaaaaaaaaagcctggtgagactttcttcatgtgttcctgtagctctgatgagtgcaatgacaacatcatcttctcagaagaatataacaccagcaatcctgacaccggtggtggagtcgagtgcccaccgtgcccagcaccacctgtggcaggaccgtcagtcttcctcttccccccaaaacccaaggacaccctcatgatctcccggacccctgaggtcacgtgcgtggtggtggacgtgagccacgaagaccccgaggtccagttcaactggtacgtggacggcgtggaggtgcataatgccaagacaaagccacgggaggagcagttcaacagcacgttccgtgtggtcagcgtcctcaccgtcgtgcaccaggactggctgaacggcaaggagtacaagtgcaaggtctccaacaaaggcctcccagcccccatcgagaaaaccatctccaaaaccaaagggcagccccgagaaccacaggtgtacaccctgcccccatcccgggaggagatgaccaagaaccaggtcagcctgacctgcctggtcaaaggcttctaccccagcgacatcgccgtggagtgggagagcaatgggcagccggagaacaactacaagaccacacctcccatgctggactccgacggctccttcttcctctacagcaagctcaccgtggacaagagcaggtggcagcaggggaacgtcttctcatgctccgtgatgcatgaggctctgcacaaccactacacgcagaagagcctctccctgtctccgggtaaa

SEQ ID NO: 3 - protein, 101 aa, Homo sapiens
QLCKFCDVRFSTCDNQKSCMSNCSITSICEKPQEVCVAVWRKNDENITLETVCHDPKLPYHDFILEDAASPKCIMKEKKKPGETFFMCSCSSDECNDNIIF

SEQ ID NO: 4 - protein, 101 aa, Homo sapiens; identical to SEQ ID NO: 3

SEQ ID NO: 5 - protein, 79 aa, Homo sapiens
ALQCFCHLCTKDNFTCVTDGLCFVSVTETTDKVIHNSMCIAEIDLIPRDRPFVCAPSSKTGSVTTTYCCNQDHCNKIEL

SEQ ID NO: 6 - protein, 25 aa, Artificial Sequence
  Description of Artificial Sequence: Synthetic peptide
PFKVAGNNDTVIMDNNVSKQVHPPI

SEQ ID NO: 7 - protein, 10 aa, Artificial Sequence
  Description of Artificial Sequence: Synthetic peptide
DPNSTNYEES

SEQ ID NO: 8 - protein, 50 aa, Artificial Sequence
  Description of Artificial Sequence: Synthetic polypeptide
PFKVAGNNDTVIMDNNIHRLPHATRNCSPCIIEDKQAEMEVDSKQVHPPI

SEQ ID NO: 9 - protein, 8 aa, Artificial Sequence
  Description of Artificial Sequence: Synthetic peptide
TAGPLLAA

SEQ ID NO: 10 - protein, 14 aa, Artificial Sequence
  Description of Artificial Sequence: Synthetic peptide
EVPGLGPSSKVTTP

SEQ ID NO: 11 - protein, 7 aa, Artificial Sequence
  Description of Artificial Sequence: Synthetic peptide
ESRGLIA

SEQ ID NO: 12 - protein, 21 aa, Artificial Sequence
  Description of Artificial Sequence: Synthetic peptide
INYYPPKPTVPNSTPQTVEME

SEQ ID NO: 13 - protein, 8 aa, Artificial Sequence
  Description of Artificial Sequence: Synthetic peptide
TEAEGRGS

SEQ ID NO: 14 - protein, 17 aa, Artificial Sequence
  Description of Artificial Sequence: Synthetic peptide
TPATPPPEYTVEPGGAE

SEQ ID NO: 15 - protein, 31 aa, Artificial Sequence
  Description of Artificial Sequence: Synthetic polypeptide
DEPALTVGNESKKQDSDSKMGTGHLMSDLNQ

SEQ ID NO: 16 - protein, 13 aa, Artificial Sequence
  Description of Artificial Sequence: Synthetic peptide
RISGDFFPGIVVP

SEQ ID NO: 17 - protein, 101 aa, Artificial Sequence
  Description of Artificial Sequence: Synthetic polypeptide
FIINDNCEDSSCSCMFFTEGPKKKEKMICKPSAADELIFDHYPLKPDHCVTELTINEDNKRWVAVCVEQPKECISTISCNSMCSKQNDCTSFRVDCFKCLQ

SEQ ID NO: 18 - protein, 101 aa, Artificial Sequence; identical to SEQ ID NO: 17
  Description of Artificial Sequence: Synthetic polypeptide

SEQ ID NO: 19 - protein, 79 aa, Artificial Sequence
  Description of Artificial Sequence: Synthetic polypeptide
LEIKNCHDQNCCYTTTVSGTKSSPACVFPRDRPILDIEAICMSNHIVKDTTETVSVFCLGDTVCTFNDKTCLHCFCQLA

SEQ ID NO: 20 - protein, 92 aa, Artificial Sequence
  Description of Artificial Sequence: Synthetic polypeptide
PFYSFKENCMNGECCCFYVEPSDKKEVCDTRDYCNIDDLWCGQKVIEISGSINKWTAFCHRRKDKDGYCPEVGTQNTRDKEWNANFFLCEQT

SEQ ID NO: 21 - protein, 108 aa, Artificial Sequence
  Description of Artificial Sequence: Synthetic polypeptide
TPATPPPEYTVEPGGAEPLHTFRENCFNGECCCFYVQPNEETAVCEQRDYCNFDDLWCGKKVLEITGSSNRWSAYCHLRKDQEGECRELGSQNTRELEWNANYYICER

SEQ ID NO: 22 - protein, 98 aa, Artificial Sequence
  Description of Artificial Sequence: Synthetic polypeptide
RISGDFFPGIVVPPLTPQLYQNCLNTRCCEITRRLQAKPSDKCQFDSGEYKMCGSALTTEGQDDEEIIAFCHGNTICTNNIADDPCHGSCYCKLFPLT

SEQ ID NO: 23 - protein, 35 aa, Artificial Sequence
  Description of Artificial Sequence: Synthetic polypeptide
PFKVAGNNDTVIMDNNVSKQVHPPIDPNSTNYEES

SEQ ID NO: 24 - protein, 60 aa, Artificial Sequence
  Description of Artificial Sequence: Synthetic polypeptide
PFKVAGNNDTVIMDNNIHRLPHATRNCSPCIIEDKQAEMEVDSKQVHPPIDPNSTNYEES

SEQ ID NO: 25 - protein, 25 aa, Artificial Sequence
  Description of Artificial Sequence: Synthetic peptide
TEAEGRGSTPATPPPEYTVEPGGAE

SEQ ID NO: 26 - protein, 44 aa, Artificial Sequence
  Description of Artificial Sequence: Synthetic polypeptide
DEPALTVGNESKKQDSDSKMGTGHLMSDLNQRISGDFFPGIVVP

SEQ ID NO: 27 - protein, 44 aa, Artificial Sequence
  Description of Artificial Sequence: Synthetic polypeptide
DEPALTVGNESKKQDSDSKMGTGHLMSDLNGRISGDFFPGIVVP

SEQ ID NO: 28 - protein, 35 aa, Artificial Sequence
  Description of Artificial Sequence: Synthetic polypeptide
PFKVAGNNDTVIMDNNVSKQVHPPGDPNSTNYEES

SEQ ID NO: 29 - protein, 25 aa, Artificial Sequence
  Description of Artificial Sequence: Synthetic peptide
TEAEGRGSTPATPPPEGTVEPGGAE

SEQ ID NO: 30 - protein, 60 aa, Artificial Sequence
  Description of Artificial Sequence: Synthetic polypeptide
PFKVAGNNDTVIMDNNIHRLPHATRNCSPCIIEDKQAEMEVDSKQVHRGGDPNSTNYEES

SEQ ID NO: 31 - protein, 35 aa, Artificial Sequence
  Description of Artificial Sequence: Synthetic polypeptide
PFKVAGNNDTVIMDNNVSKQVHPGGDPNSTNYEES

SEQ ID NO: 32 - protein, 35 aa, Artificial Sequence
  Description of Artificial Sequence: Synthetic polypeptide
PFKVAGNNDTVIMDNNVSKQVHRGGDPNSTNYEES

SEQ ID NO: 33 - protein, 60 aa, Artificial Sequence
  Description of Artificial Sequence: Synthetic polypeptide
PFKVAGNNDTVIMDNNIHRLPHATRNCSPCIIEDKQAEMGGGSGGGSGGGSPNSTNYEES

SEQ ID NO: 34 - protein, 35 aa, Artificial Sequence
  Description of Artificial Sequence: Synthetic polypeptide
PFKVAGNNDTVIMDNNVSKGGSGGGSPNSTNYEES

SEQ ID NO: 35 - protein, 35 aa, Artificial Sequence
  Description of Artificial Sequence: Synthetic polypeptide
PFKVAGNNDTVIMDGGGSGGGSGGGSPNSTNYEES

SEQ ID NO: 36 - protein, 60 aa, Artificial Sequence
  Description of Artificial Sequence: Synthetic polypeptide
PFKVAGNNDTVIMDNNGGSGGGSGGGSGGGSGGGSGGGSGGGSKQVHPPIDPNSTNYEES

SEQ ID NO: 37 - protein, 60 aa, Artificial Sequence
  Description of Artificial Sequence: Synthetic polypeptide
PFKVAGNNDTVIMDNNGGSGGGSGGGSGGGSGGGSGGGSGGGSGGGSGGGDPNSTNYEES

SEQ ID NO: 38 - protein, 35 aa, Artificial Sequence; identical to SEQ ID NO: 23
  Description of Artificial Sequence: Synthetic polypeptide

SEQ ID NO: 39 - protein, 48 aa, Artificial Sequence
  Description of Artificial Sequence: Synthetic polypeptide
PFKVAGNNDIVIMDNNVSKQVHPPIMDNNVSKQVHPPIDPNSTNYEES

SEQ ID NO: 40 - protein, 32 aa, Artificial Sequence
  Description of Artificial Sequence: Synthetic polypeptide
PFKVAGNNDTVIMDNNVSKQVHPPNSTNYEES

SEQ ID NO: 41 - protein, 43 aa, Artificial Sequence
  Description of Artificial Sequence: Synthetic polypeptide
PFKVAGNNDIVIMDNNVSKQVHPPIGGGGGGGGDPNSTNYEES

SEQ ID NO: 42 - protein, 47 aa, Artificial Sequence
  Description of Artificial Sequence: Synthetic polypeptide
PFKVAGNNDTVIMDNNVSKQVHPPISGGGSGGGSGGGDPNSTNYEES

SEQ ID NO: 43 - protein, 60 aa, Artificial Sequence; identical to SEQ ID NO: 24
  Description of Artificial Sequence: Synthetic polypeptide

SEQ ID NO: 44 - protein, 53 aa, Artificial Sequence
  Description of Artificial Sequence: Synthetic polypeptide
PFKVAGNNDTVIMDNNIHRLPHATREDKQAEMEVDSKQVHPPIDPNSTNYEES

SEQ ID NO: 45 - protein, 25 aa, Artificial Sequence
  Description of Artificial Sequence: Synthetic peptide
TEAEGRGSTPATPPPEYTVEPGGAE

SEQ ID NO: 46 - protein, 35 aa, Artificial Sequence
  Description of Artificial Sequence: Synthetic polypeptide
TEAEGRGSGGGGGGGGGGTPATPPPEYTVEPGGAE

SEQ ID NO: 47 - protein, 44 aa, Artificial Sequence; identical to SEQ ID NO: 26
  Description of Artificial Sequence: Synthetic polypeptide

SEQ ID NO: 48 - protein, 40 aa, Artificial Sequence
  Description of Artificial Sequence: Synthetic polypeptide
DEPALTVGNESKKQDSDSKMGTGHSDLNQRISGDPGIVVP

SEQ ID NO: 49 - DNA, 20 bp, Artificial Sequence
  Description of Artificial Sequence: Synthetic primer
tgagtggctgtcttttgacg

SEQ ID NO: 50 - DNA, 20 bp, Artificial Sequence
  Description of Artificial Sequence: Synthetic primer
ttctctgtggagctgaagca

SEQ ID NO: 51 - DNA, 20 bp, Artificial Sequence
  Description of Artificial Sequence: Synthetic primer
cacgcctctcttgtttcctc

SEQ ID NO: 52 - DNA, 20 bp, Artificial Sequence
  Description of Artificial Sequence: Synthetic primer
ttttccaagggcaatgaaag

SEQ ID NO: 53 - DNA, 20 bp, Artificial Sequence
  Description of Artificial Sequence: Synthetic primer
gaaggctgcactcaggaaac

SEQ ID NO: 54 - DNA, 20 bp, Artificial Sequence
  Description of Artificial Sequence: Synthetic primer
gctgcttggctatgtgttca

SEQ ID NO: 55 - DNA, 20 bp, Artificial Sequence
  Description of Artificial Sequence: Synthetic primer
ctttatcctgggtctccctg

SEQ ID NO: 56 - DNA, 20 bp, Artificial Sequence
  Description of Artificial Sequence: Synthetic primer
tgatgcctccctgacataca

SEQ ID NO: 57 - DNA, 18 bp, Artificial Sequence
  Description of Artificial Sequence: Synthetic primer
aataatctgggtaaggcc

SEQ ID NO: 58 - DNA, 22 bp, Artificial Sequence
  Description of Artificial Sequence: Synthetic primer
gcagaacgaacgcaacctatca

SEQ ID NO: 59 - DNA, 21 bp, Artificial Sequence
  Description of Artificial Sequence: Synthetic primer
tggacgaacagcaggtgaacg

SEQ ID NO: 60 - DNA, 21 bp, Artificial Sequence
  Description of Artificial Sequence: Synthetic primer
gcactgatctcgccgttcagg

SEQ ID NO: 61 - DNA, 20 bp, Artificial Sequence
  Description of Artificial Sequence: Synthetic primer
tgtcaccaactgggacgata

SEQ ID NO: 62 - DNA, 20 bp, Artificial Sequence
  Description of Artificial Sequence: Synthetic primer
accctcatagatgggcacag

SEQ ID NO: 63 - protein, 137 aa, Homo sapiens
TIPPHVQKSVNNDMIVTDNNGAVKFPQLCKFCDVRFSTCDNQKSCMSNCSITSICEKPQEVCVAVWRKNDENITLETVCHDPKLPYHDFILEDAASPKCIMKEKKKPGETFFMCSCSSDECNDNIIFSEEYNTSNPD

SEQ ID NO: 64 - protein, 222 aa, Homo sapiens
ECPPCPAPPVAGPSVFLFPPKPKDTLMISRTPEVTCVVVDVSHEDPEVQFNWYVDGVEVHNAKTKPREEQFNSTFRVVSVLTVVHQDWLNGKEYKCKVSNKGLPAPIEKTISKTKGQPREPQVYTLPPSREEMTKNQVSLTCLVKGFYPSDIAVEWESNGQPENNYKTTPPMLDSDGSFFLYSKLTVDKSRWQQGNVFSCSVMHEALHNHYTQKSLSLSPGK

SEQ ID NO: 65 - protein, 15 aa, Homo sapiens
EPKSCDKTHTCPPCP

SEQ ID NO: 66 - protein, 12 aa, Homo sapiens
ERKCCVECPPCP

SEQ ID NO: 67 - protein, 62 aa, Homo sapiens
ELKTPLGDTTHTCPRCPEPKSCDTPPPCPRCPEPKSCDTPPPCPRCPEPKSCDTPPPCPRCP

SEQ ID NO: 68 - protein, 12 aa, Homo sapiens
ESKYGPPCPSCP

SEQ ID NO: 69 - protein, 217 aa, Homo sapiens
APELLGGPSVFLFPPKPKDTLMISRTPEVTCVVVDVSHEDPEVKFNWYVDGVEVHNAKTKPREEQYNSTYRVVSVLTVLHQDWLNGKEYKCKVSNKALPAPIEKTISKAKGQPREPQVYTLPPSRDELTKNQVSLTCLVKGFYPSDIAVEWESNGQPENNYKTTPPVLDSDGSFFLYSKLTVDKSRWQQGNVFSCSVMHEALHNHYTQKSLSLSPGK

SEQ ID NO: 70 - protein, 216 aa, Homo sapiens
APPVAGPSVFLFPPKPKDTLMISRTPEVTCVVVDVSHEDPEVQFNWYVDGVEVHNAKTKPREEQFNSTFRVVSVLTVVHQDWLNGKEYKCKVSNKGLPAPIEKTISKTKGQPREPQVYTLPPSREEMTKNQVSLTCLVKGFYPSDIAVEWESNGQPENNYKTTPPMLDSDGSFFLYSKLTVDKSRWQQGNVFSCSVMHEALHNHYTQKSLSLSPGK

SEQ ID NO: 71 - protein, 217 aa, Homo sapiens
APELLGGPSVFLFPPKPKDTLMISRTPEVTCVVVDVSHEDPEVQFKWYVDGVQVHNAKTKPREQQFNSTFRVVSVLTVLHQNWLDGKEYKCKVSNKALPAPIEKTISKTKGQPREPQVYTLPPSREEMTKNQVSLTCLVKGFYPSDIAVEWESSGQPENNYNTTPPMLDSDGSFFLYSKLTVDKSRWQQGNIFSCSVMHEALHNRFTQKSLSLSPGK

SEQ ID NO: 72 - protein, 217 aa, Homo sapiens
APEFLGGPSVFLFPPKPKDTLMISRTPEVTCVVVDVSQEDPEVQFNWYVDGVEVHNAKTKPREEQFNSTYRVVSVLTVLHQDWLNGKEYKCKVSNKGLPSSIEKTISKAKGQPREPQVYTLPPSQEEMTKNQVSLTCLVKGFYPSDIAVEWESNGQPENNYKTTPPVLDSDGSFFLYSRLTVDKSRWQEGNVFSCSVMHEALHNHYTQKSLSLSLGK

SEQ ID NO: 73 - protein, 107 aa, Homo sapiens
GVQVETISPGDGRTFPKRGQTCVVHYTGMLEDGKKFDSSRDRNKPFKFMLGKQEVIRGWEEGVAQMSVGQRAKLTISPDYAYGATGHPGIIPPHATLVFDVELLKLE

SEQ ID NO: 74 - protein, 342 aa, Homo sapiens
EDPSLDRPFISEGTTLKDLIYDMTTSGSGSGLPLLVQRTIARTIVLQESIGKGRFGEVWRGKWRGEEVAVKIFSSREERSWFREAEIYQTVMLRHENILGFIAADNKDNGTWTQLWLVSDYHEHGSLFDYLNRYTVTVEGMIKLALSTASGLAHLHMEIVGTQGKPAIAHRDLKSKNILVKKNGTCCIADLGLAVRHDSATDTIDIAPNHRVGTKRYMAPEVLDDSINMKHFESFKRADIYAMGLVFWEIARRCSIGGIHEDYQLPYYDLVPSDPSVEEMRKVVCEQKLRPNIPNRWQSCEALRVMAKIMRECWYANGAARLTALRIKKTLSQLSQQEGIKM

SEQ ID NO: 75 - protein, 785 aa, Homo sapiens
MTSHYVIAIFALMSSCLATAGPEPGALCELSPVSASHPVQALMESFTVLSGCASRGTTGLPQEVHVLNLRTAGQGPGQLQREVTLHLNPISSVHIHHKSVVFLLNSPHPLVWHLKTERLATGVSRLFLVSEGSVVQFSSANFSLTAETEERNFPHGNEHLLNWARKEYGAVTSFTELKIARNIYIKVGEDQVFPPKCNIGKNFLSLNYLAEYLQPKAAEGCVMSSQPQNEEVHIIELITPNSNPYSAFQVDITIDIRPSQEDLEVVKNLILILKCKKSVNWVIKSFDVKGSLKIIAPNSIGFGKESERSMTMTKSIRDDIPSTQGNLVKWALDNGYSPITSYTMAPVANRFHLRLENNEEMGDEEVHTIPPELRILLDPGALPALQNPPIRGGEGQNGGLPFPFPDISRRVWNEEGEDGLPRPKDPVIPSIQLFPGLREPEEVQGSVDIALSVKCDNEKMIVAVEKDSFQASGYSGMDVTLLDPTCKAKMNGTHFVLESPLNGCGTRPRWSALDGVVYYNSIVIQVPALGDSSGWPDGYEDLESGDNGFPGDMDEGDASLFTRPEIVVFNCSLQQVRNPSSFQEQPHGNITFNMELYNTDLFLVPSQGVFSVPENGHVYVEVSVTKAEQELGFAIQTCFISPYSNPDRMSHYTIIENICPKDESVKFYSPKRVHFPIPQADMDKKRFSFVFKPVFNTSLLFLQCELTLCTKMEKHPQKLPKCVPPDEACTSLDASIIWAMMQNKKTFTKPLAVIHHEAESKEKGPSMKEPNPISPPIFHGLDTLT

SEQ ID NO: 76 - DNA, 23 bp, Artificial Sequence
  Description of Artificial Sequence: Synthetic primer
aagcttgccgccgccatgggtcg

SEQ ID NO: 77 - DNA, 23 bp, Artificial Sequence
  Description of Artificial Sequence: Synthetic primer
ctggaattcgtcaggattgctgg

SEQ ID NO: 78 - protein, 477 aa, Homo sapiens
MGRGLLRGLWPLHIVLWTRIASTIPPHVQKSVNNDMIVTDNNGAVKFPQLCKFCDVRFSTCDNQKSCMSNCSITSICEKPQEVCVAVWRKNDENITLETVCHDPKLPYHDFILEDAASPKCIMKEKKKPGETFFMCSCSSDECNDNIIFSEEYNTSNPDLLLVIFQVTGISLLPPLGVAISVIIIFYCYRVNRQQKLSSTWETGKTRKLMEFSEHCAIILEDDRSDISSTCANNINHNTELLPIELDTLVGKGRFAEVYKAKLKQNTSEQFETVAVKIFPYEEYASWKTEKDIFSDINLKHENILQFLTAEERKTELGKQYWLITAFHAKGNLQEYLTRHVISWEDLRKLGSSLARGIAHLHSDHTPCGRPKMPIVHRDLKSSNILVKNDLTCCLCDFGLSLRLDPTLSVDDLANSGQVGTARYMAPEVLESRMNLENVESFKQTDVYSMALVLWEMTSRCNAVGEVKDYEPPFGSK

SEQ ID NO: 79 - protein, 4 aa, Artificial Sequence
  Description of Artificial Sequence: Synthetic peptide
TGGG